European Patent Application EP 4 317 441 A1, published February 7, 2024. Title: Novel Recombinant Mycobacterium smegmatis and Use Thereof. Applicant: CLIPS BnC. The sequence listing filed with the application follows.

SEQUENCE LISTING (6 sequences)

SEQ ID NO: 1 - DNA, 6412 bp, Artificial Sequence
  pMyong2 plasmid
agcgcccaatacgcaaaccgcctctccccgcgcgttggccgattcattaatgcagctggcacgacaggtttcccgactggaaagcgggcagtgagcgcaacgcaattaatgtgagttagctcactcattaggcaccccaggctttacactttatgcttccggctcgtatgttgtgtggaattgtgagcggataacaatttcacacaggaaacagctatgaccatgattacgccaagcttggtaccgagctcggatccactagtaacggccgccagtgtgctggaattcgcccttaagcttaggcgggcaacacgacatctcaatagttggcacggagctcctaaacgacgacagccccgctaatgcggggccgcaacgtcgatttggctctacttcgtctctggagtttcgtctctggagtttcaggtccgagcggctaactcggtcctaggcgtctcccgtgccgcgcccccgaagggacagtcttgctggactggtctcacggtagcgcatacccgaatcagattcgtggtgacgcgcaaaaccgtgatctcacatttacagattcccgtgcatccgtgtgcacggattcacgcccatctgggcattcacgtggccgttttggtgcctccgtctgggctctcgtcgctcccggcggcgcgtcgtggtgacaaccgcgttcgacgcggcagagattgccgccgcggtcccggaatctggctcaccgtgcagcggtacagcgtcagctcgactgcgcagaatccgcgccaaggaagcccgcagggcgtcgatcgaacgctgtggggcggtgccggccgcggtgccgatgtggtcgtcgcgggagttgtggactgccgatctgcgggtgcttttgtcgggtccggagttcagcacgcgccgggtgatttcggcggcgacggtgctcgctgtcgcggtggcgatggccgagttcgccgaccatgccacgggccgcaatgtggcggtgacaaacgaggttctggccgagcgcgcgaggtgttctaagcgttcggtgaccgcggcgcgcggggtgttgaaagcgttgggtgtcgcggtggaagcggtacgtgggcatggctctgcgaccacacacacggtcggtaatcgaccgagcatttggcacctggtaagccgacgccagcccaccatcgacaacccgcccacggccccgcagaacggccgcggcgagcctgccgatacggtgcccgatcgcggccagagcgcgcccgtggctgtggagacttgcgacctaccaccatcccgtagggataggtgggtaactcctgttgagaattactcaccaagcacgcgcgagcgcgcgagcgcggaaaattcttccccaaaacaaacacaaccggcgcggtcgcggcggcgctaccgcgccacgccgcgccccctggacgttcagcgactcgccgccggcctggtcacgccggcagtcggccacggcccagacaacgacgggcggcgaaccgcgctgatcgccggcctggagcagggccatatcggggccatctgcgacgcgatcacgacggccggcatcgacgcgaccgcctggactccgaagacgctcacggcggcactgaacgccgacgcgcgggtgaccggctggtcgtggccggatcgcatcgaacgtcctggcgcgttcctggcgtcgcggctgcgccgcctgcccgcacggcccgacaccagtggcccggttgacaacggcctggatcaggcccgtaggacacccgttgagccgtcagcggcccgtgtagcgccggtacagacggccgctggccgcgcgtacgcccgtgcgttgttcgccgagcagcgacggcaccgggtgaccgccgccaatgcccagtcagccgcggtgccggtgcgccaaagtgcgccagaaaccgcggtgtgcgcaacgtgcggatgctcggacgcaccacggcggcggttcctgccaacgcggcgggctcacatttgcgatgcctgtttccaaggatgtggtggtgggcaggcgcgtactggtcgcgtcggaacggtcggcagcagttccgcggtgccacagtgccagtagtcgggcagggcttgcacggggatgcggacccatccgccggccgcggccggcgatgggtccagtgtcgcgttagggccgtcgtccagccgcgccagctcgcggtcggatgcgatcagcttggcaccgtagatgtcgtcgtggcggcggtcccacgtgttggtgatgcggtcgcggtaccagcctgtccagtcttcgccggtgccgccggcggtgagcccggcccggtaccacgcttcgaggcgatcacggccccgtgcgtggttgatggtctgggccgcagcccagtccgcgtcacggagggctctgtcggcttcgtccatgaacccgcgccgggtcatgtcgatgatggctggcgacggggcgtcgtaggggcctggcatgggcggaggcagtcggaactgttgcggtttgcttgcgttcagttcctcgtcctgctggtgggtgcggtcgtgcagggcaaggctgtcgcggtaccaggcgtcgagcgcggtgcgccagtccccgccagtggcgtagggctcccacggttgcggtggcagggtggtgaactcgtgcaggaccaggccgtcgatgtcgtcgcgcagttcttcaccggcgatggcggcgatgcgggcgcagtagccgggcagatggctacgccagtcggcgggcagttcgccgctgcgcgcccaccgcagcacatcggcccacaacccccatggaagggcgaattctgcagatatccatcacactggcggccgctcgagcatgcatctagagggcccaattcgccctatagtgagtcgtattacaattcactggccgtcgttttacaacgtcgtgactgggaaaaccctggcgttacccaacttaatcgccttgcagcacatccccctttcgccagctggcgtaatagcgaagaggcccgcaccgatcgcccttcccaacagttgcgcagcctgaatggcgaatggacgcgccctgtagcggcgcattaagcgcggcgggtgtggtggttacgcgcagcgtgaccgctacacttgccagcgccctagcgcccgctcctttcgctttcttcccttcctttctcgccacgttcgccggctttccccgtcaagctctaaatcgggggctccctttagggttccgatttagtgctttacggcacctcgaccccaaaaaacttgattagggtgatggttcacgtagtgggccatcgccctgatagacggtttttcgccctttgacgttggagtccacgttctttaatagtggactcttgttccaaactggaacaacactcaaccctatctcggtctattcttttgatttataagggattttgccgatttcggcctattggttaaaaaatgagctgatttaacaaaaatttaacgcgaattttaacaaaattcagggcgcaagggctgctaaaggaagcggaacacgtagaaagccagtccgcagaaacggtgctgaccccggatgaatgtcagctactgggctatctggacaagggaaaacgcaagcgcaaagagaaagcaggtagcttgcagtgggcttacatggcgatagctagactgggcggttttatggacagcaagcgaaccggaattgccagctggggcgccctctggtaaggttgggaagccctgcaaagtaaactggatggctttcttgccgccaaggatctgatggcgcaggggatcaagatctgatcaagagacaggatgaggatcgtttcgcatgattgaacaagatggattgcacgcaggttctccggccgcttgggtggagaggctattcggctatgactgggcacaacagacaatcggctgctctgatgccgccgtgttccggctgtcagcgcaggggcgcccggttctttttgtcaagaccgacctgtccggtgccctgaatgaactgcaggacgaggcagcgcggctatcgtggctggccacgacgggcgttccttgcgcagctgtgctcgacgttgtcactgaagcgggaagggactggctgctattgggcgaagtgccggggcaggatctcctgtcatcccaccttgctcctgccgagaaagtatccatcatggctgatgcaatgcggcggctgcatacgcttgatccggctacctgcccattcgaccaccaagcgaaacatcgcatcgagcgagcacgtactcggatggaagccggtcttgtcgatcaggatgatctggacgaagagcatcaggggctcgcgccagccgaactgttcgccaggctcaaggcgcgcatgcccgacggcgaggatctcgtcgtgacccatggcgatgcctgcttgccgaatatcatggtggaaaatggccgcttttctggattcatcgactgtggccggctgggtgtggcggaccgctatcaggacatagcgttggctacccgtgatattgctgaagagcttggcggcgaatgggctgaccgcttcctcgtgctttacggtatcgccgctcccgattcgcagcgcatcgccttctatcgccttcttgacgagttcttctgaattgaaaaaggaagagtatgagtattcaacatttccgtgtcgcccttattcccttttttgcggcattttgccttcctgtttttgctcacccagaaacgctggtgaaagtaaaagatgctgaagatcagttgggtgcacgagtgggttacatcgaactggatctcaacagcggtaagatccttgagagttttcgccccgaagaacgttttccaatgatgagcacttttaaagttctgctatgtggcgcggtattatcccgtattgacgccgggcaagagcaactcggtcgccgcatacactattctcagaatgacttggttgagtactcaccagtcacagaaaagcatcttacggatggcatgacagtaagagaattatgcagtgctgccataaccatgagtgataacactgcggccaacttacttctgacaacgatcggaggaccgaaggagctaaccgcttttttgcacaacatgggggatcatgtaactcgccttgatcgttgggaaccggagctgaatgaagccataccaaacgacgagcgtgacaccacgatgcctgtagcaatggcaacaacgttgcgcaaactattaactggcgaactacttactctagcttcccggcaacaattaatagactggatggaggcggataaagttgcaggaccacttctgcgctcggcccttccggctggctggtttattgctgataaatctggagccggtgagcgtgggtctcgcggtatcattgcagcactggggccagatggtaagccctcccgtatcgtagttatctacacgacggggagtcaggcaactatggatgaacgaaatagacagatcgctgagataggtgcctcactgattaagcattggtaactgtcagaccaagtttactcatatatactttagattgatttaaaacttcatttttaatttaaaaggatctaggtgaagatcctttttgataatctcatgaccaaaatcccttaacgtgagttttcgttccactgagcgtcagaccccgtagaaaagatcaaaggatcttcttgagatcctttttttctgcgcgtaatctgctgcttgcaaacaaaaaaaccaccgctaccagcggtggtttgtttgccggatcaagagctaccaactctttttccgaaggtaactggcttcagcagagcgcagataccaaatactgttcttctagtgtagccgtagttaggccaccacttcaagaactctgtagcaccgcctacatacctcgctctgctaatcctgttaccagtggctgctgccagtggcgataagtcgtgtcttaccgggttggactcaagacgatagttaccggataaggcgcagcggtcgggctgaacggggggttcgtgcacacagcccagcttggagcgaacgacctacaccgaactgagatacctacagcgtgagctatgagaaagcgccacgcttcccgaagggagaaaggcggacaggtatccggtaagcggcagggtcggaacaggagagcgcacgagggagcttccagggggaaacgcctggtatctttatagtcctgtcgggtttcgccacctctgacttgagcgtcgatttttgtgatgctcgtcaggggggcggagcctatggaaaaacgccagcaacgcggcctttttacggttcctggccttttgctggccttttgctcacatgttctttcctgcgttatcccctgattctgtggataaccgtattaccgcctttgagtgagctgataccgctcgccgcagccgaacgaccgagcgcagcgagtcagtgagcgaggaagcggaag

SEQ ID NO: 2 - DNA, 2469 bp, Mycobacterium intracellulare
aggcgggcaacacgacatctcaatagttggcacggagctcctaaacgacgacagccccgctaatgcggggccgcaacgtcgatttggctctacttcgtctctggagtttcgtctctggagtttcaggtccgagcggctaactcggtcctaggcgtctcccgtgccgcgcccccgaagggacagtcttgctggactggtctcacggtagcgcatacccgaatcagattcgtggtgacgcgcaaaaccgtgatctcacatttacagattcccgtgcatccgtgtgcacggattcacgcccatctgggcattcacgtggccgttttggtgcctccgtctgggctctcgtcgctcccggcggcgcgtcgtggtgacaaccgcgttcgacgcggcagagattgccgccgcggtcccggaatctggctcaccgtgcagcggtacagcgtcagctcgactgcgcagaatccgcgccaaggaagcccgcagggcgtcgatcgaacgctgtggggcggtgccggccgcggtgccgatgtggtcgtcgcgggagttgtggactgccgatctgcgggtgcttttgtcgggtccggagttcagcacgcgccgggtgatttcggcggcgacggtgctcgctgtcgcggtggcgatggccgagttcgccgaccatgccacgggccgcaatgtggcggtgacaaacgaggttctggccgagcgcgcgaggtgttctaagcgttcggtgaccgcggcgcgcggggtgttgaaagcgttgggtgtcgcggtggaagcggtacgtgggcatggctctgcgaccacacacacggtcggtaatcgaccgagcatttggcacctggtaagccgacgccagcccaccatcgacaacccgcccacggccccgcagaacggccgcggcgagcctgccgatacggtgcccgatcgcggccagagcgcgcccgtggctgtggagacttgcgacctaccaccatcccgtagggataggtgggtaactcctgttgagaattactcaccaagcacgcgcgagcgcgcgagcgcggaaaattcttccccaaaacaaacacaaccggcgcggtcgcggcggcgctaccgcgccacgccgcgccccctggacgttcagcgactcgccgccggcctggtcacgccggcagtcggccacggcccagacaacgacgggcggcgaaccgcgctgatcgccggcctggagcagggccatatcggggccatctgcgacgcgatcacgacggccggcatcgacgcgaccgcctggactccgaagacgctcacggcggcactgaacgccgacgcgcgggtgaccggctggtcgtggccggatcgcatcgaacgtcctggcgcgttcctggcgtcgcggctgcgccgcctgcccgcacggcccgacaccagtggcccggttgacaacggcctggatcaggcccgtaggacacccgttgagccgtcagcggcccgtgtagcgccggtacagacggccgctggccgcgcgtacgcccgtgcgttgttcgccgagcagcgacggcaccgggtgaccgccgccaatgcccagtcagccgcggtgccggtgcgccaaagtgcgccagaaaccgcggtgtgcgcaacgtgcggatgctcggacgcaccacggcggcggttcctgccaacgcggcgggctcacatttgcgatgcctgtttccaaggatgtggtggtgggcaggcgcgtactggtcgcgtcggaacggtcggcagcagttccgcggtgccacagtgccagtagtcgggcagggcttgcacggggatgcggacccatccgccggccgcggccggcgatgggtccagtgtcgcgttagggccgtcgtccagccgcgccagctcgcggtcggatgcgatcagcttggcaccgtagatgtcgtcgtggcggcggtcccacgtgttggtgatgcggtcgcggtaccagcctgtccagtcttcgccggtgccgccggcggtgagcccggcccggtaccacgcttcgaggcgatcacggccccgtgcgtggttgatggtctgggccgcagcccagtccgcgtcacggagggctctgtcggcttcgtccatgaacccgcgccgggtcatgtcgatgatggctggcgacggggcgtcgtaggggcctggcatgggcggaggcagtcggaactgttgcggtttgcttgcgttcagttcctcgtcctgctggtgggtgcggtcgtgcagggcaaggctgtcgcggtaccaggcgtcgagcgcggtgcgccagtccccgccagtggcgtagggctcccacggttgcggtggcagggtggtgaactcgtgcaggaccaggccgtcgatgtcgtcgcgcagttcttcaccggcgatggcggcgatgcgggcgcagtagccgggcagatggctacgccagtcggcgggcagttcgccgctgcgcgcccaccgcagcacatcggcccacaaccc

SEQ ID NO: 3 - DNA, 375 bp, Artificial Sequence
  hsp65 promoter
ggtgaccacaacgacgcgcccgctttgatcggggacgtctgcggccgaccatttacgggtcttgttgtcgttggcggtcatgggccgaacatactcacccggatcggagggccgaggacaaggtcgaacgaggggcatgacccggtgcggggcttcttgcactcggcataggcgagtgctaagaataacgttggcactcgcgaccggtgagtcgtaggtcgggacggtgaggccaggcccgtcgtcgcagcgagtggcagcgaggacaacttgagccgtccgtcgcgggcactgcgcccggccagcgtaagtagcggggttgccgtcacccggtgacccccggtttcatccccgatccggaggaatcacttcgca

SEQ ID NO: 4 - DNA, 345 bp, Artificial Sequence
  TB optimized human MIF
atgccgatgttcatcgtgaacaccaacgtgccgcgcgcctcggtgccggacggcttcctgtcggagctgacccagcagctggcccaggccaccggcaagccgccgcagtacatcgccgtgcacgtggtgccggaccagctgatggccttcggcggctcgtcggagccgtgcgccctgtgctcgctgcactcgatcggcaagatcggcggcgcccagaaccgctcgtactcgaagctgctgtgcggcctgctggccgagcgcctgcgcatctcgccggaccgcgtgtacatcaactactacgacatgaacgccgccaacgtgggctggaacaactcgaccttcgcc

SEQ ID NO: 5 - DNA, 462 bp, Artificial Sequence
  TB optimized human IL-7
atggactgcgacatcgagggcaaggacggcaagcagtacgagtcggtgctgatggtgtcgatcgaccagctgctggactcgatgaaggagatcggctcgaactgcctgaacaacgagttcaacttcttcaagcgccacatctgcgacgccaacaaggagggcatgttcctgttccgcgccgcccgcaagctgcgccagttcctgaagatgaactcgaccggcgacttcgacctgcacctgctgaaggtgtcggagggcaccaccatcctgctgaactgcaccggccaggtgaagggccgcaagccggccgccctgggcgaggcccagccgaccaagtcgctggaggagaacaagtcgctgaaggagcagaagaagctgaacgacctgtgcttcctgaagcgcctgctgcaggagatcaagacctgctggaacaagatcctgatgggcaccaaggagcactaa

SEQ ID NO: 6 - DNA, 7565 bp, Artificial Sequence
  pMyong2-hMIF::hIL7
agcgcccaatacgcaaaccgcctctccccgcgcgttggccgattcattaatgcagctggcacgacaggtttcccgactggaaagcgggcagtgagcgcaacgcaattaatgtgagttagctcactcattaggcaccccaggctttacactttatgcttccggctcgtatgttgtgtggaattgtgagcggataacaatttcacacaggaaacagctatgaccatgattacgccaagcttggtaccgagctcggatccactagtaacggccgccagtgtgctggaattcgcccttaagcttaggcgggcaacacgacatctcaatagttggcacggagctcctaaacgacgacagccccgctaatgcggggccgcaacgtcgatttggctctacttcgtctctggagtttcgtctctggagtttcaggtccgagcggctaactcggtcctaggcgtctcccgtgccgcgcccccgaagggacagtcttgctggactggtctcacggtagcgcatacccgaatcagattcgtggtgacgcgcaaaaccgtgatctcacatttacagattcccgtgcatccgtgtgcacggattcacgcccatctgggcattcacgtggccgttttggtgcctccgtctgggctctcgtcgctcccggcggcgcgtcgtggtgacaaccgcgttcgacgcggcagagattgccgccgcggtcccggaatctggctcaccgtgcagcggtacagcgtcagctcgactgcgcagaatccgcgccaaggaagcccgcagggcgtcgatcgaacgctgtggggcggtgccggccgcggtgccgatgtggtcgtcgcgggagttgtggactgccgatctgcgggtgcttttgtcgggtccggagttcagcacgcgccgggtgatttcggcggcgacggtgctcgctgtcgcggtggcgatggccgagttcgccgaccatgccacgggccgcaatgtggcggtgacaaacgaggttctggccgagcgcgcgaggtgttctaagcgttcggtgaccgcggcgcgcggggtgttgaaagcgttgggtgtcgcggtggaagcggtacgtgggcatggctctgcgaccacacacacggtcggtaatcgaccgagcatttggcacctggtaagccgacgccagcccaccatcgacaacccgcccacggccccgcagaacggccgcggcgagcctgccgatacggtgcccgatcgcggccagagcgcgcccgtggctgtggagacttgcgacctaccaccatcccgtagggataggtgggtaactcctgttgagaattactcaccaagcacgcgcgagcgcgcgagcgcggaaaattcttccccaaaacaaacacaaccggcgcggtcgcggcggcgctaccgcgccacgccgcgccccctggacgttcagcgactcgccgccggcctggtcacgccggcagtcggccacggcccagacaacgacgggcggcgaaccgcgctgatcgccggcctggagcagggccatatcggggccatctgcgacgcgatcacgacggccggcatcgacgcgaccgcctggactccgaagacgctcacggcggcactgaacgccgacgcgcgggtgaccggctggtcgtggccggatcgcatcgaacgtcctggcgcgttcctggcgtcgcggctgcgccgcctgcccgcacggcccgacaccagtggcccggttgacaacggcctggatcaggcccgtaggacacccgttgagccgtcagcggcccgtgtagcgccggtacagacggccgctggccgcgcgtacgcccgtgcgttgttcgccgagcagcgacggcaccgggtgaccgccgccaatgcccagtcagccgcggtgccggtgcgccaaagtgcgccagaaaccgcggtgtgcgcaacgtgcggatgctcggacgcaccacggcggcggttcctgccaacgcggcgggctcacatttgcgatgcctgtttccaaggatgtggtggtgggcaggcgcgtactggtcgcgtcggaacggtcggcagcagttccgcggtgccacagtgccagtagtcgggcagggcttgcacggggatgcggacccatccgccggccgcggccggcgatgggtccagtgtcgcgttagggccgtcgtccagccgcgccagctcgcggtcggatgcgatcagcttggcaccgtagatgtcgtcgtggcggcggtcccacgtgttggtgatgcggtcgcggtaccagcctgtccagtcttcgccggtgccgccggcggtgagcccggcccggtaccacgcttcgaggcgatcacggccccgtgcgtggttgatggtctgggccgcagcccagtccgcgtcacggagggctctgtcggcttcgtccatgaacccgcgccgggtcatgtcgatgatggctggcgacggggcgtcgtaggggcctggcatgggcggaggcagtcggaactgttgcggtttgcttgcgttcagttcctcgtcctgctggtgggtgcggtcgtgcagggcaaggctgtcgcggtaccaggcgtcgagcgcggtgcgccagtccccgccagtggcgtagggctcccacggttgcggtggcagggtggtgaactcgtgcaggaccaggccgtcgatgtcgtcgcgcagttcttcaccggcgatggcggcgatgcgggcgcagtagccgggcagatggctacgccagtcggcgggcagttcgccgctgcgcgcccaccgcagcacatcggcccacaacccccatggaagggcgaattctgcagatatcggtgaccacaacgacgcgcccgctttgatcggggacgtctgcggccgaccatttacgggtcttgttgtcgttggcggtcatgggccgaacatactcacccggatcggagggccgaggacaaggtcgaacgaggggcatgacccggtgcggggcttcttgcactcggcataggcgagtgctaagaataacgttggcactcgcgaccggtgagtcgtaggtcgggacggtgaggccaggcccgtcgtcgcagcgagtggcagcgaggacaacttgagccgtccgtcgcgggcactgcgcccggccagcgtaagtagcggggttgccgtcacccggtgacccccggtttcatccccgatccggaggaatcacttcgcaatgccgatgttcatcgtgaacaccaacgtgccgcgcgcctcggtgccggacggcttcctgtcggagctgacccagcagctggcccaggccaccggcaagccgccgcagtacatcgccgtgcacgtggtgccggaccagctgatggccttcggcggctcgtcggagccgtgcgccctgtgctcgctgcactcgatcggcaagatcggcggcgcccagaaccgctcgtactcgaagctgctgtgcggcctgctggccgagcgcctgcgcatctcgccggaccgcgtgtacatcaactactacgacatgaacgccgccaacgtgggctggaacaactcgaccttcgccatggactgcgacatcgagggcaaggacggcaagcagtacgagtcggtgctgatggtgtcgatcgaccagctgctggactcgatgaaggagatcggctcgaactgcctgaacaacgagttcaacttcttcaagcgccacatctgcgacgccaacaaggagggcatgttcctgttccgcgccgcccgcaagctgcgccagttcctgaagatgaactcgaccggcgacttcgacctgcacctgctgaaggtgtcggagggcaccaccatcctgctgaactgcaccggccaggtgaagggccgcaagccggccgccctgggcgaggcccagccgaccaagtcgctggaggagaacaagtcgctgaaggagcagaagaagctgaacgacctgtgcttcctgaagcgcctgctgcaggagatcaagacctgctggaacaagatcctgatgggcaccaaggagcactaatctagagggcccaattcgccctatagtgagtcgtattacaattcactggccgtcgttttacaacgtcgtgactgggaaaaccctggcgttacccaacttaatcgccttgcagcacatccccctttcgccagctggcgtaatagcgaagaggcccgcaccgatcgcccttcccaacagttgcgcagcctgaatggcgaatggacgcgccctgtagcggcgcattaagcgcggcgggtgtggtggttacgcgcagcgtgaccgctacacttgccagcgccctagcgcccgctcctttcgctttcttcccttcctttctcgccacgttcgccggctttccccgtcaagctctaaatcgggggctccctttagggttccgatttagtgctttacggcacctcgaccccaaaaaacttgattagggtgatggttcacgtagtgggccatcgccctgatagacggtttttcgccctttgacgttggagtccacgttctttaatagtggactcttgttccaaactggaacaacactcaaccctatctcggtctattcttttgatttataagggattttgccgatttcggcctattggttaaaaaatgagctgatttaacaaaaatttaacgcgaattttaacaaaattcagggcgcaagggctgctaaaggaagcggaacacgtagaaagccagtccgcagaaacggtgctgaccccggatgaatgtcagctactgggctatctggacaagggaaaacgcaagcgcaaagagaaagcaggtagcttgcagtgggcttacatggcgatagctagactgggcggttttatggacagcaagcgaaccggaattgccagctggggcgccctctggtaaggttgggaagccctgcaaagtaaactggatggctttcttgccgccaaggatctgatggcgcaggggatcaagatctgatcaagagacaggatgaggatcgtttcgcatgattgaacaagatggattgcacgcaggttctccggccgcttgggtggagaggctattcggctatgactgggcacaacagacaatcggctgctctgatgccgccgtgttccggctgtcagcgcaggggcgcccggttctttttgtcaagaccgacctgtccggtgccctgaatgaactgcaggacgaggcagcgcggctatcgtggctggccacgacgggcgttccttgcgcagctgtgctcgacgttgtcactgaagcgggaagggactggctgctattgggcgaagtgccggggcaggatctcctgtcatcccaccttgctcctgccgagaaagtatccatcatggctgatgcaatgcggcggctgcatacgcttgatccggctacctgcccattcgaccaccaagcgaaacatcgcatcgagcgagcacgtactcggatggaagccggtcttgtcgatcaggatgatctggacgaagagcatcaggggctcgcgccagccgaactgttcgccaggctcaaggcgcgcatgcccgacggcgaggatctcgtcgtgacccatggcgatgcctgcttgccgaatatcatggtggaaaatggccgcttttctggattcatcgactgtggccggctgggtgtggcggaccgctatcaggacatagcgttggctacccgtgatattgctgaagagcttggcggcgaatgggctgaccgcttcctcgtgctttacggtatcgccgctcccgattcgcagcgcatcgccttctatcgccttcttgacgagttcttctgaattgaaaaaggaagagtatgagtattcaacatttccgtgtcgcccttattcccttttttgcggcattttgccttcctgtttttgctcacccagaaacgctggtgaaagtaaaagatgctgaagatcagttgggtgcacgagtgggttacatcgaactggatctcaacagcggtaagatccttgagagttttcgccccgaagaacgttttccaatgatgagcacttttaaagttctgctatgtggcgcggtattatcccgtattgacgccgggcaagagcaactcggtcgccgcatacactattctcagaatgacttggttgagtactcaccagtcacagaaaagcatcttacggatggcatgacagtaagagaattatgcagtgctgccataaccatgagtgataacactgcggccaacttacttctgacaacgatcggaggaccgaaggagctaaccgcttttttgcacaacatgggggatcatgtaactcgccttgatcgttgggaaccggagctgaatgaagccataccaaacgacgagcgtgacaccacgatgcctgtagcaatggcaacaacgttgcgcaaactattaactggcgaactacttactctagcttcccggcaacaattaatagactggatggaggcggataaagttgcaggaccacttctgcgctcggcccttccggctggctggtttattgctgataaatctggagccggtgagcgtgggtctcgcggtatcattgcagcactggggccagatggtaagccctcccgtatcgtagttatctacacgacggggagtcaggcaactatggatgaacgaaatagacagatcgctgagataggtgcctcactgattaagcattggtaactgtcagaccaagtttactcatatatactttagattgatttaaaacttcatttttaatttaaaaggatctaggtgaagatcctttttgataatctcatgaccaaaatcccttaacgtgagttttcgttccactgagcgtcagaccccgtagaaaagatcaaaggatcttcttgagatcctttttttctgcgcgtaatctgctgcttgcaaacaaaaaaaccaccgctaccagcggtggtttgtttgccggatcaagagctaccaactctttttccgaaggtaactggcttcagcagagcgcagataccaaatactgttcttctagtgtagccgtagttaggccaccacttcaagaactctgtagcaccgcctacatacctcgctctgctaatcctgttaccagtggctgctgccagtggcgataagtcgtgtcttaccgggttggactcaagacgatagttaccggataaggcgcagcggtcgggctgaacggggggttcgtgcacacagcccagcttggagcgaacgacctacaccgaactgagatacctacagcgtgagctatgagaaagcgccacgcttcccgaagggagaaaggcggacaggtatccggtaagcggcagggtcggaacaggagagcgcacgagggagcttccagggggaaacgcctggtatctttatagtcctgtcgggtttcgccacctctgacttgagcgtcgatttttgtgatgctcgtcaggggggcggagcctatggaaaaacgccagcaacgcggcctttttacggttcctggccttttgctggccttttgctcacatgttctttcctgcgttatcccctgattctgtggataaccgtattaccgcctttgagtgagctgataccgctcgccgcagccgaacgaccgagcgcagcgagtcagtgagcgaggaagcggaag